European Patent Application EP 4 714 465 A1, published March 25, 2026. Title: 针对猫FIPV构建环状RNA和疫苗的方法. Applicant: 北京合生基因科技有限公司. Application CN. The sequence listing filed with the application follows.

SEQUENCE LISTING (48 sequences)

SEQ ID NO: 1 - protein, 245 aa, synthetic construct
ERYCAMQNTGSQCINGTDSSCSTCFERGGLIWHLANWNFSWSVILIVFITVLKYGRPQFSWLVYGIKMLIMWLLWPIVLALTIFNAYSEYQVSRYVMFGFSVAGAVVTFALWMMYFVRSIQLYRRTKSWWSFNPETNAILCVNALGRSYVLPLDGTPTGVTLTLLSGNLYAEGFKMAGGLTIEHLPKYVMIATPSRTIVYTLVGKQLKATTATGWAYYVKSKAGDYSTEARTDNLSEHEKLLHMV

SEQ ID NO: 2 - protein, 375 aa, synthetic construct
ATQGQRVNWGDEPSKRRGRSNSRGRKNNTIPLSFFNPIQLEPGSKFWSVCPRDFVPKGIGNKDQQIGYWNRQERYRIVKGQRKELPERWFFYFLGTGPQADAKFKDKIDGVFWVAKDGAMNKPTTLGTRGTNNESKPLKFDGKIPPQFQLEVNRSRNNSRSGSQSRSVSRNRSQSRGRQQSNNQNNVEDTIVAVLQKLGVTEKQRSRSKSRDRGDSKPRDTTPNNANKHTWKKTAGKGDVTNFYGARSASANFGDSDLVANGNAAKSYPQIAECVPSVSSMLFGSQWSAEDDGDQVKVTLTHTYYLPKDDAKTSQFLEQIDAYKRPSQVAKDQRQRKSRSKSAEKKPEELSVTLVEAYTDVFDDTQVEMIDEVTN

SEQ ID NO: 3 - protein, 1433 aa, synthetic construct
TTNNECIQVNVTQLAGNENLIRDFLFSNFKEEGSVVVGGYYPTEVWYNCSRTARTTAFQYFNNIHAFYFVMEAMENSTGNARGKPLLFHVHGEPVSVIISAYRDDVQQRPLLKHGLVCITKNRHINYEQFTSNQWNSTCTGADRKIPFSVIPTDNGTKIYGLEWNDDFVTAYISGRSYHLNINTNWFNNVTLLYSRSSTATWEYSAAYAYQGVSNFTYYKLNNTNGLKTYELCEDYEHCTGYATNVFAPTSGGYIPDGFSFNNWFLLTNSSTFVSGRFVTNQPLLINCLWPVPSFGVAAQEFCFEGAQFSQCNGVSLNNTVDVIRFNLNFTADVQSGMGATVFSLNTTGGVILEISCYSDTVSESSSYSYGEIPFGITDGPRYCYVLYNGTALKYLGTLPPSVKEIAISKWGHFYINGYNFFSTFPIGCISFNLTTGVSGAFWTIAYTSYTEALVQVENTAIKNVTYCNSHINNIKCSQLTANLNNGFYPVASSEVGFVNKSVVLLPSFFTYTAVNITIDLGMKLSGYGQPIASTLSNITLPMQDNNTDVYCIRSNQFSVYVHSTCKSSLWDNIFNQDCTDVLEATAVIKTGTCPFSFDKLNNYLTFNKFCLSLSPVGANCKFDVAARTRTNEQVVRSLYVIYEEGDNIVGVPSDNSGLHDLSVLHLDSCTDYNIYGRTGVGIIRRTNSTLLSGLYYTSLSGDLLGFKNVSDGVIYSVTPCDVSAQAAVIDGAIVGAMTSINSELLGLTHWTTTPNFYYYSIYNYTSERTRDTAIDSNDVDCEPVITYSNIGVCKNGALVFINVTHSDGDVQPISTGNVTIPTNFTISVQVEYMQVYTTPVSIDCARYVCNGNPRCNKLLTQYVSACQTIEQALAMGARLENMEVDSMLFVSENALKLASVEAFNSTENLDSIYKEWPSIGGSWLGGLKDILPSHNSKRKYGSAIEDLLFDKVVTSGLGTVDEDYKRCTGGYDIADLVCAQYYNGIMVLPGVANADKMTMYTASLAGGITLGALGGGAVAIPFAVAVQARLNYVALQTDVLNKNQQILANAFNQAIGNITQAFGKVNDAIHQTSQGLATVAKALAKVQDVVNTQGQALSHLTVQLQNNFQAISSSISDIYNRLDPPSADAQVDRLITGRLTALNAFVSQTLTRQAEVRASRQLAKDKVNECVRSQSQRFGFCGNGTHLFSLANAAPNGMIFFHTVLLPTAYETVTAWSGICASDGDRTFGLVVKDVQLTLFRNLDDKFYLTPRTMYQPRVATSSDFVQIEGCDVLFVNATVIDLPSIIPDYIDINQTVQDILENYRPNWTVPEFTLDIFNATYLNLTGEIDDLEFRSEKLHNTTVELAILIDNINNTLVNLEWLNRIETYVKWPWYVWLLIGLVVVFCIPLLLFCCFSTGCCGCIGCLGSCCHSICSRRQFENYEPIEKVHVH

SEQ ID NO: 4 - DNA, 735 bp, synthetic construct
  source 1..735: mol_type = other DNA
gaacgctactgtgccatgcaaaatacaggctcgcagtgcattaatggcacagattcatcatgtagcacctgttttgaacgtggtggtcttatttggcatctggctaactggaacttcagctggtctgtaatattgattgtttttataacagtgttaaaatatggaagaccgcaattcagctggctcgtttatggcattaaaatgctgatcatgtggctattatggcctattgttctagcgcttacgatttttaatgcatactctgagtaccaagtttccagatatgtaatgttcggctttagtgttgcaggtgcagttgtaacgtttgcactatggatgatgtattttgtgagatctattcagctgtatagacggaccaaatcatggtggtcttttaatcctgaaaccaatgcgattctttgtgtcaatgcattgggtagaagctatgtactccctcttgatggcactcctacaggtgttactcttaccctactttcaggaaatctatacgctgaaggttttaaaatggctggtggtcttaccatcgagcatttgcctaaatatgtcatgattgctacgcctagtagaaccatcgtttacacattagttggaaaacaactaaaggcaactactgccactggatgggcttactatgtaaaatctaaagctggtgattactcaacagaagcacgtactgataatttgagtgaacatgaaaaattattacatatggtg

SEQ ID NO: 5 - DNA, 735 bp, synthetic construct
  source 1..735: mol_type = other DNA
gagagatactgtgccatgcagaacacaggcagccagtgcatcaatggaacagacagcagctgcagcacctgctttgaaagaggaggcctgatctggcacctggccaactggaacttcagctggagtgtgatcctgattgtcttcattacagtgctgaagtacggcaggccccagttcagctggctggtgtacggcatcaagatgctcatcatgtggctgctgtggcccattgtgttggccctcaccatcttcaatgcctacagcgagtaccaggtgtccagatacgtgatgttcggcttctcagtggcaggagccgtggtgacctttgccctctggatgatgtactttgtgaggtccatccagctctacagaagaacaaagagctggtggagcttcaacccagaaaccaacgccatcctgtgtgtcaatgccctgggcagatcctatgtgctgcccctggatggcacccccacaggcgtcaccctcaccctcctgagcggcaacctgtacgccgagggcttcaagatggccggcggcctgacaatcgagcacctgcccaagtatgtgatgattgccacccccagcaggacaatagtctacaccctggtgggaaaacagctgaaggctaccacagccacaggctgggcctactacgtcaagagcaaggccggcgactacagcacagaggccaggaccgacaacctgtccgaacatgaaaaactcctgcacatggtc

SEQ ID NO: 6 - DNA, 735 bp, synthetic construct
  source 1..735: mol_type = other DNA
gagaggtactgcgccatgcagaacacaggctcccagtgcatcaacggaacagactcctcctgcagcacctgcttcgagagaggaggcctcatttggcacctggccaactggaacttcagctggtcagtcattctgatagtcttcataacagtgctgaagtacggcaggccccagttctcctggctcgtgtatggcatcaagatgctgatcatgtggctgctgtggcccatcgtcctggccctgaccatcttcaacgcctactcagagtaccaggtcagcaggtacgtgatgttcggcttctccgtggccggagcagtggtgaccttcgccctgtggatgatgtacttcgtgaggagcatccaactgtacaggaggaccaaaagctggtggtccttcaacccagaaaccaacgccatcctctgcgtgaacgccctgggcaggtcctacgtcctccccctggacggcacccccaccggggtcaccctcaccctcctgtcagggaacctgtacgctgagggcttcaagatggctggaggcctgacaattgaacacctgcccaagtacgtcatgatcgcaacaccctccagaaccatcgtctacaccctggtgggcaagcagctgaaggccaccaccgccaccggctgggcctactacgtcaagtccaaggccggcgactacagcaccgaggccaggaccgacaacctctcagagcacgagaagctgctgcacatggtg

SEQ ID NO: 7 - DNA, 735 bp, synthetic construct
  source 1..735: mol_type = other DNA
gagaggtactgtgccatgcagaacaccggttcccagtgcatcaacggcacagactcctcctgctccacctgcttcgagagaggaggcctgatctggcacctggcaaactggaacttcagctggagcgtgatcctgatagtgttcataaccgtcctgaagtacggcagaccacagttctcatggcttgtctatggcatcaagatgctgattatgtggctgctttggcctatcgtcctggccctgaccatcttcaacgcctactctgagtaccaggtgtcaaggtatgtcatgttcggcttctcagtggctggagctgtggtgacctttgctctgtggatgatgtacttcgtgaggtccatccagctgtacaggaggacaaagtcatggtggtccttcaacccagaaaccaatgccatcctgtgcgtcaacgcactgggcagaagctacgtcctaccactggacggcactcctacaggagtgaccctgaccctgctgtcaggcaatctgtacgcagaggggttcaagatggccggtggcctgaccatcgagcatctgcctaagtacgtgatgatcgccacccctagcaggacaatcgtgtacaccctggtgggaaagcagctaaaggcgaccacagccacaggctgggcctactacgtgaagtccaaggcaggggactattcaaccgaggccaggaccgacaacctgtcagagcacgagaagctgctgcacatggtc

SEQ ID NO: 8 - DNA, 1125 bp, synthetic construct
  source 1..1125: mol_type = other DNA
gccacacagggacaacgcgtcaactggggagatgaaccttccaaaagacgtggtcgttctaactctcgtggtcggaagaataacactatacctctttcattcttcaatcccatccaactcgaaccaggatcaaaattttggagcgtatgtccgagagattttgttcccaagggaataggtaacaaggatcaacaaattggttattggaatagacaagagcgttaccgcattgtcaaaggtcagcgtaaggaacttcctgagaggtggtttttctacttcttaggcacaggacctcaagctgatgctaaatttaaagacaagattgatggagtcttctgggttgcaaaggatggtgccatgaataaaccaacaacacttggcactcgtggtaccaacaatgaatccaaaccactgaaatttgatggtaagataccaccgcaatttcagcttgaagtgaaccgatctaggaacaactcaagaagtggttctcagtctagatctgtctctagaaacaggtctcaatccagaggaagacaacaatccaataatcagaataatgttgaggatacaattgtagctgtgcttcagaaattaggtgttactgaaaagcaaaggtcacgttctaaatctagagatcgtggtgactctaaacctagagacacaacacctaataatgccaacaaacacacctggaagaagactgcaggtaaaggtgatgtgacaaatttctatggtgctagaagtgcttcagctaactttggtgatagtgatctcgttgccaacggtaacgctgccaaatcctaccctcagatagctgaatgcgttccatcagtgtctagcatgctcttcggtagtcaatggtctgctgaagatgatggtgatcaagtgaaagtcacgctcactcatacctattacctgccaaaagatgatgccaaaaccagccaattcctagaacagattgacgcttacaagcggccatctcaagtggctaaagatcagaggcaaagaaaatctcgttctaagtctgctgagaagaagcctgaggaattgtctgtaactcttgtagaggcatatacggatgtgtttgatgacacacaggttgagatgattgatgaggttacgaac

SEQ ID NO: 9 - DNA, 1125 bp, synthetic construct
  source 1..1125: mol_type = other DNA
gccacacagggccagagggtgaactggggcgacgagccatccaagaggaggggaaggagcaacagcagaggaaggaagaacaacaccatccccctgtccttcttcaacccaattcagctagagccaggcagcaagttctggtcagtgtgccccagagacttcgtgcccaagggcatcggaaacaaggaccagcagatcggctactggaacagacaggagagatacagaattgtgaaaggccagagaaaggagctgccagagaggtggttcttctacttcctgggcaccggcccacaggcagacgccaagttcaaggacaagatcgatggagtgttctgggtggccaaggacggcgccatgaacaagcccaccacactgggcacaagaggaacaaacaatgagagcaagccactgaagtttgatggcaagatcccaccccagttccagctggaggtgaacaggagcagaaacaacagcagaagcggcagccagagcagaagtgtgagcagaaacagaagccagagcagaggaagacagcagagcaacaaccagaacaacgtggaggacaccatcgtggccgtgctgcagaagctgggggtcacagaaaagcagaggagcagaagcaagagcagggacagaggagacagcaagccaagagacaccacccccaacaacgccaacaagcacacctggaagaagacagccggcaagggagatgtgaccaacttctacggcgccagaagcgccagcgccaacttcggagactcagacctggtggccaatggaaacgcagccaagagctacccccagatcgcagagtgtgtgccctctgtctccagcatgctgtttggcagccagtggagcgccgaggacgacggtgaccaggtgaaggtgaccctgacacacacatactacctgcccaaagatgacgccaagaccagccagttcctggagcagattgatgcctacaagaggcccagccaggtggccaaggaccagagacagaggaagagcaggtccaagagcgccgagaagaagccagaagaattgagtgtcaccctggtggaggcctacacagacgtgtttgatgacacccaggtggagatgattgatgaggtgaccaac

SEQ ID NO: 10 - DNA, 1125 bp, synthetic construct
  source 1..1125: mol_type = other DNA
gccacccagggccagagagtgaactggggcgacgagccctcaaaaaggaggggcagatccaacagcagaggcaggaagaacaacaccatccccctgagcttcttcaaccccatccagctggagccaggctccaagttctggtcagtgtgcccaagggacttcgtgcccaagggcatcggcaacaaggaccagcagatcggctactggaacaggcaggagagatacagaatcgtgaagggccagaggaaggaactgccagaaaggtggttcttctacttcctgggcaccggcccccaggctgacgccaagttcaaagacaagatcgacggggtgttctgggtggccaaggacggcgccatgaacaagccaacaacactgggcaccagaggaaccaacaacgagagcaagccactgaagtttgacggcaagatccccccccagttccagctggaagtcaacaggagcaggaacaacagcaggtccggctcacaaagcaggagcgtgtccagaaacagatcccagtcaagaggaagacagcagtccaacaaccagaacaacgtggaggacaccatagtggccgtgctgcagaagctgggagtcacagagaagcagaggagcagatccaagtccagggacaggggagacagcaagcccagggacaccacacccaacaacgccaacaagcacacctggaagaagacagccggcaagggagatgtgaccaacttctacggcgccagaagcgcctcagccaacttcggagactcagacctggtggccaacggaaacgccgccaagagctacccccagatcgccgaatgtgtcccctcagtgtcctccatgctcttcggctcacagtggtcagcagaggacgacggcgaccaggtgaaggtgaccctgacccacacctactacctgcccaaggacgacgccaagacaagccagttcctggagcagatcgacgcctacaagaggccatcccaggtggccaaggaccagaggcagaggaagagcagaagcaagtcagccgagaagaaaccagaggagctgtcagtcaccctggtggaggcctacaccgacgtgttcgacgacacccaggtggagatgatcgacgaggtgaccaac

SEQ ID NO: 11 - DNA, 1125 bp, synthetic construct
  source 1..1125: mol_type = other DNA
gcaacacaaggacagagagtaaattggggggatgagcccagcaagaggcgaggcagaagcaactcaagagggagaaaaaacaataccatcccactgtcattcttcaaccccattcaactggagccaggctctaaattctggagtgtatgccccagggactttgtgcccaagggcatagggaacaaggaccagcaaataggatactggaaccggcaggagagatacagaattgtcaagggtcagagaaaggagctgccagagagatggttcttctacttcctaggaacaggcccacaggcagacgctaagttcaaggataagatcgatggtgtcttctgggtcgccaaggatggtgcaatgaataaaccaaccaccctggggaccagggggacaaacaatgagtccaagcccctcaagtttgatggcaaaatccccccacagttccagctggaggtcaacaggagcaggaacaatagccgttcagggtcccagtccagatctgtgtccagaaacaggtcccagagcaggggacggcagcagagtaacaaccagaataatgtggaagacaccatagtagcagtgctccagaaactgggggtcacagaaaaacagaggagcaggtccaagtctagggaccgtggggactctaagccaagggacaccacacccaacaacgccaacaagcacacatggaaaaaaacagcagggaagggtgatgtcaccaacttttacggggccaggtcagcctctgcaaacttcggggatagtgacctggtggccaacggcaatgctgctaaatcctaccctcagattgctgagtgcgtaccctctgtatcctctatgctctttggctcacaatggtctgctgaggatgatggtgaccaggtcaaggtcaccttgacccatacctactatctgcccaaggatgatgcaaaaaccagccagttcctagagcagatagatgcctacaagaggcccagccaggtggccaaggatcagaggcagagaaagagcagatccaagagcgcagaaaagaaaccagaggagttatctgtgaccctggtggaggcctacacagatgtctttgatgatacacaggtggaaatgatagatgaggtgactaac

SEQ ID NO: 12 - DNA, 4302 bp, synthetic construct
  source 1..4302: mol_type = other DNA
acaacaaataatgaatgcatacaagttaacgtaacacaattggctggcaatgaaaaccttatcagagattttctgtttagtaactttaaagaagaaggaagtgtagttgttggtggttattaccctacagaggtgtggtacaactgctctagaacagctcgaactactgcctttcagtattttaataatatacatgccttttattttgttatggaagccatggaaaatagcactggtaatgcacgtggtaaaccattattatttcatgtgcatggtgagcctgttagtgttattatatcggcttatagggatgatgtgcaacaaaggccccttttaaaacatgggttagtgtgcataactaaaaatcgccatattaactatgaacaattcacctccaaccagtggaattccacatgtacgggtgctgacagaaaaattcctttctctgtcatacccacggacaatggaacaaaaatctatggtcttgagtggaatgatgactttgttacagcttatattagtggtcgttcttatcacttgaacatcaatactaattggtttaacaatgtcacacttttgtattcacgctcaagcactgctacctgggaatacagtgctgcatatgcttaccaaggtgtttctaacttcacttattacaagttaaataacaccaatggtctaaaaacctatgaattatgtgaagattatgaacattgcactggctatgctaccaatgtatttgctccgacatcaggtggttacatacctgatggatttagttttaacaattggttcttgcttacaaatagttccacttttgttagtggcaggtttgtaacaaatcaaccattattgattaattgcttgtggccagtgcccagttttggtgtagcagcacaagaattttgttttgaaggtgcacagtttagccaatgtaatggtgtgtctttaaataacacagtggatgttattagattcaaccttaatttcactgcagatgtacaatctggtatgggtgctacagtattttcactgaatacaacaggtggtgtcattcttgaaatttcatgttatagtgacacagtgagtgagtctagttcttacagttatggtgaaatcccgttcggcataactgacggaccacgatactgttatgtactttacaatggcacagctcttaaatatttaggaacattaccacccagtgtaaaggaaattgctattagtaagtggggccatttttatattaatggttacaatttctttagcacatttcctattggttgtatatcttttaatttaaccactggtgttagtggagctttttggacaattgcttacacatcgtatactgaagcattagtacaagttgaaaacacagctattaaaaatgtgacgtattgtaacagtcacattaataacattaaatgttctcaacttactgctaatttgaataatggattttatcctgttgcttcaagtgaagtaggtttcgttaataagagtgttgtgttattacctagctttttcacatacaccgctgtcaatataaccattgatcttggtatgaagcttagtggttatggtcaacccatagcctcgacactaagtaacatcacactaccaatgcaggataacaatactgatgtgtactgtattcgttctaaccaattctcagtttatgttcattccacttgcaaaagttctttatgggacaatatttttaatcaagactgcacggatgttttagaggctacagctgttataaaaactggtacttgtcctttctcatttgataaattgaacaattacttgacttttaacaagttctgtttgtcgttgagtcctgttggtgctaattgcaagtttgatgttgctgcacgtacaagaaccaatgagcaggttgttagaagtctatatgtaatatatgaagaaggagacaacatagtgggtgtaccgtctgataatagcggtctgcacgatttgtctgtgctacacctagactcctgtacagattacaatatatatggtagaactggtgttggtattattagacgaactaacagtacgctacttagtggcttatattacacatcactatcaggtgatttgttaggctttaaaaatgttagtgatggtgtcatttattctgtgacgccatgtgatgtaagcgcacaagcggctgttattgatggtgccatagttggagctatgacttccattaacagtgaactgttaggtctaacacattggacaacgacacctaatttttattactactctatatataattacacaagtgagaggactcgtggcactgcaattgacagtaacgatgttgattgtgaacctgtcataacctattctaatataggtgtttgtaaaaatggtgctttggtttttattaacgtcacacattctgacggagacgtgcaaccaattagcactggtaatgtcacgatacctacaaattttactatatctgtgcaagttgaatacatgcaggtttacactacaccagtatcaatagattgtgcaagatacgtttgtaatggtaaccctagatgtaacaaattgttaacacaatatgtgtctgcatgtcaaactattgaacaagcacttgcaatgggtgccagacttgaaaacatggaggttgattccatgttgtttgtctcggaaaatgcccttaaattggcatctgttgaggcgttcaatagtacagaaaatttagatcctatttacaaagaatggcctagcataggtggttcttggctaggaggtctaaaagatatactaccgtcccataatagcaaacgtaagtatggttctgctatagaagatttgctttttgataaagttgtaacatctggtttaggtacagttgatgaagattataaacgttgtactggtggttacgacatagcagacttggtgtgtgctcaatattacaatggcatcatggttctaccaggtgtagctaatgctgacaagatgactatgtacacagcatcacttgcaggtggtataacattaggtgcacttggtggtggcgccgtggctataccttttgcagtagcagtacaggctagacttaattatgttgctctacaaactgatgtattgaataaaaaccaacagatcctggctaatgctttcaatcaagctattggtaacattacacaggcttttggtaaggttaatgatgctatacatcaaacatcacaaggtcttgccactgttgctaaagcgttggcaaaagtgcaagatgttgtcaacacacaagggcaagctttaagtcaccttacagtacaattgcaaaataattttcaagccattagtagttctattagtgatatttataacaggcttgacgaactgagtgctgatgcacaagttgataggctgattacaggtagacttacagcacttaatgcatttgtgtctcagactctaaccagacaagcagaggttagggctagtagacaacttgccaaagacaaggttaatgaatgtgttaggtctcagtctcagagattcggattctgtggtaatggtacacatttgttttcactagcaaatgcagcaccaaatggcatgattttctttcatacagtactattaccaacagcttatgaaactgtaacagcttggtcaggtatttgtgcttcagatggcgatcgcactttcggacttgtcgttaaagatgtgcagttgacgttgtttcgtaatctagatgacaagttctatttgacccccagaactatgtatcagcctagagttgcaactagttctgattttgttcaaattgaagggtgtgatgtgttgtttgtcaacgcgactgtaattgatttgcctagtattatacctgactatattgacattaatcaaactgttcaagacatattagaaaattacagaccaaactggactgtacctgaatttacacttgatattttcaacgcaacctatttaaatctgactggtgaaattgatgacttagagtttaggtcagaaaagctacataacactacagtagaacttgccattctcattgataacattaataatacattagtcaatcttgaatggctcaatagaattgaaacttatgtaaaatggccttggtatgtgtggctactgataggtttagtagtagtattttgcataccattactgctattttgctgttttagcacaggttgttgtggatgcataggttgtttaggaagttgttgtcactctatatgtagtagaagacaatttgaaaattatgaaccaattgaaaaagtgcatgtccactaa

SEQ ID NO: 13 - DNA, 4299 bp, synthetic construct
  source 1..4299: mol_type = other DNA
accaccaacaatgaatgcatccaggtgaacgtgacccagctggcaggcaatgaaaatttgatcagagacttcctgttcagcaacttcaaggaggagggcagtgtagtggtgggaggctactacccaacagaggtgtggtacaactgcagcagaacagccagaaccacagccttccagtacttcaacaacatccacgccttctactttgtgatggaggccatggaaaacagcacaggaaatgccagaggaaaacccctgctcttccacgtgcacggagagcccgtgtcagtcatcatcagcgcctacagagatgacgtccagcagcggcccctgctgaagcatggactggtctgcatcaccaagaacagacacatcaactacgagcagttcaccagcaaccagtggaacagcacctgcacaggagcagacagaaaaatccccttcagcgtcatccccacagacaacggcaccaaaatctatggcctggagtggaatgatgactttgtgacagcctatatcagcggcaggagctaccacctcaacatcaacaccaactggttcaacaacgtcaccctgctctactccagatccagcacagccacctgggagtacagcgccgcctatgcctaccagggagtctccaacttcacctactacaaactgaacaacaccaacggcctgaaaacctacgagctgtgtgaggactacgagcactgcacaggctatgccacaaatgtgtttgccccaaccagcggaggctacatcccagacggcttctccttcaacaactggttcctcctcaccaactcctccacatttgtgagcggcagatttgtgaccaaccagcccctgctgatcaactgcctgtggcccgtgcccagctttggagtggcagcccaggagttctgcttcgagggagcccagttcagccagtgcaacggagtcagcctgaacaacacagtggacgtgatcagattcaacctgaacttcacagcagacgtgcagagtggaatgggagccaccgtcttcagcctgaacaccacaggaggagtgatcctggagatcagctgctacagcgacacagtgagcgagagcagcagctacagctacggagagatcccatttggcatcacagatggccccaggtactgctacgtcctgtacaatggaacagccctgaaatacctgggcaccctcccacccagcgtgaaggagatcgccatcagcaagtggggccacttctacatcaatggctacaacttcttcagcaccttccccatcggctgcatctccttcaacctgaccacaggagtgagcggggccttctggacaatcgcctacacatcctacacagaagccctggtgcaggtggagaacacagccatcaaaaacgtcacctactgcaacagccacatcaacaacatcaagtgcagccagctgacagccaacctgaacaacggcttctacccagtggccagctcagaggtgggcttcgtgaacaagagcgtggtgctcctgcccagcttcttcacctacacagcagtgaacatcacaattgacctgggcatgaagctgagcggctacggccagccaattgccagcaccctctccaacatcaccctccccatgcaggacaataacacagatgtgtactgcatcagatccaaccagttctctgtctacgtgcacagcacctgcaaaagcagcctgtgggacaacatcttcaaccaggactgcacagatgtcctggaggccacagccgtgatcaaaacaggcacctgccccttcagctttgacaaactcaacaactaccttacattcaacaaattctgcctctccctcagcccagtgggagccaactgcaagtttgatgtggccgccaggaccaggacaaatgaacaagtggtcagaagcctctacgtcatctacgaggagggagacaacatcgtgggggtccccagcgacaacagcggcctgcacgacctgagtgtgctccacctggacagctgcacagactacaacatctacggcaggactggggtgggcatcatcagaagaaccaacagcacactgctgagtggcctgtactacaccagcctgagtggagacttgctgggcttcaagaatgtgtcagatggggtgatctacagtgtgaccccctgtgacgtgtctgcccaggctgcagtcatcgacggagccatcgtgggagccatgaccagcattaacagcgagctgctgggcctgacccactggaccaccacccccaacttctactactactccatctacaactacacatcagaaagaacaagagacacagccatcgacagcaatgacgtggactgtgagccagtcatcacctacagcaacatcggagtgtgcaagaacggagccctggtgttcatcaacgtgacccacagcgacggagatgtccagcccatcagcacaggaaatgtgaccatcccaaccaacttcaccatcagcgtccaggtggaatacatgcaggtgtacaccaccccagtgtccatcgactgtgccagatacgtgtgcaatggaaaccccagatgcaacaagctcctcacccagtacgtgtcagcctgccagacaatcgagcaggccctggccatgggagccaggctcgagaacatggaagtggacagcatgctgtttgtctcagagaatgccctgaaactggccagcgtggaggccttcaacagcacagagaacctggacagcatctacaaggagtggccatcaatcggaggcagctggctgggaggacttaaggacatcctgccaagccacaacagcaaaagaaagtacggcagcgccattgaggacctgctgtttgacaaggtggtcacctccggcctgggcacagtggatgaggactacaagagatgcaccggcggctatgacattgccgacctggtgtgtgcccagtactacaatggcatcatggtgctgcctggagtggccaacgccgacaaaatgaccatgtacaccgcctccctggctggaggcatcacactgggagccctggggggaggagcagtggccatcccctttgcagtggctgtgcaggccagactcaactacgtggccctgcagacagacgtgctcaacaagaaccagcagatcctggccaacgctttcaaccaggctatcggaaacatcacccaggcctttggaaaagtgaatgatgccatccaccagaccagccagggcctggccacagtggccaaggccctggccaaggtgcaggacgtggtcaacacccagggccaggccctcagtcacctcacagtacagctccagaacaacttccaggcaatctcctcctccatcagcgacatctacaacaggctggaccccccaagcgctgatgcccaggtggacagactgatcacaggaagactcacagccctcaacgcatttgtgtcccagacactgaccaggcaggcagaggtcagggccagcaggcagctggccaaggacaaggtgaatgagtgcgtgaggagccagagccagagatttggcttctgcggaaacggcacccacctgttcagcctggccaacgccgcccccaacggcatgattttcttccacacagtcctcctccccacagcctacgaaacagtgacagcctggtcaggcatctgtgccagcgacggagacagaacctttggcctggtggtgaaggatgtgcagctcaccctcttcagaaacctggatgacaagttctacctcaccccaagaaccatgtaccagcccagagtggccacaagcagcgactttgtgcagattgagggctgtgacgtgctgtttgtgaatgcaacagtgattgacctcccaagcatcatcccagattacatcgacatcaaccagacagtgcaggacatcctggagaactacaggcccaactggacagtgccagagttcaccctggacatcttcaacgccacctacctgaacctgacaggagaaattgacgacctggagttcagatcagaaaaacttcacaacaccaccgtggagcttgccatcctcattgacaacattaacaacacactggtcaacctggaatggctgaacagaattgaaacctacgtgaagtggccctggtatgtgtggctgctgattggactggtggtggtgttctgcatcccactgctgctgttctgctgcttcagcaccggctgctgtggatgcatcggctgcttgggcagctgctgccacagcatctgcagcaggaggcagtttgagaactacgaaccaattgaaaaagtgcacgtccac

SEQ ID NO: 14 - DNA, 4299 bp, synthetic construct
  source 1..4299: mol_type = other DNA
accaccaacaacgagtgcatccaggtgaacgtgacccagctggcaggcaacgagaacctcatcagagacttcctcttctccaacttcaaggaggagggctcagtggtggtcggcggctactacccaacagaggtgtggtacaactgctcaaggaccgccagaaccacagccttccagtacttcaacaacatccacgccttctacttcgtgatggaggccatggagaactccaccgggaacgccaggggcaagccactactcttccacgtgcacggagagccagtgagcgtgatcatctcagcctacagggacgacgtgcagcagcgccccctgctgaagcatggactggtgtgcatcaccaagaacaggcacatcaactacgagcagttcaccagcaaccagtggaacagcacctgcaccggcgcagacaggaagatccccttctcagtgatcccaacagacaacggaaccaaaatctacggcctggagtggaacgacgacttcgtgaccgcctacatcagcggcaggtcctaccatctcaacatcaacaccaactggttcaacaacgtcaccctcctctacagcaggtcatccacagccacctgggagtactcagctgcctatgcataccagggagtctccaacttcacatactacaaactcaacaacaccaacggcctcaagacctacgagctgtgtgaggactacgagcactgcaccggctacgcaacaaacgtcttcgccccaacctccggaggctacatcccagacggcttctccttcaacaactggttcctcctcacaaacagctccaccttcgtgtcaggaaggttcgtgaccaaccagcccctgctcatcaactgcctctggcccgtcccctccttcggagtggccgcccaggagttctgcttcgagggagcccagttctcccagtgcaacggagtctccctcaacaacaccgtggacgtcatcagattcaacctcaacttcacagcagacgtccagagcggcatgggagccaccgtgttcagcctgaacaccacaggaggagtgatcctggagatctcctgctactcagacacagtgtcagagtcctcctcctacagctacggagagatcccattcggcatcacagacggccccagatactgctacgtgctgtacaacggcacagccctgaagtacctgggcaccctccccccatcagtgaaggagatcgccatcagcaagtggggccacttctacatcaacggctacaacttcttctccaccttccccatcggctgcatcagcttcaacctgaccaccggagtgtccggagccttctggaccatcgcctacacatcatacaccgaggccctggtgcaggtggagaacacagccataaagaacgtgacctactgcaacagccacatcaacaacatcaagtgctcccagctgacagccaacctgaacaacggcttctacccagtggcctccagcgaggtgggcttcgtgaacaagagcgtggtcctactcccctccttcttcacctacacagcagtcaacatcacaattgacctgggcatgaagctgtccggctacggccagccaatcgccagcaccctgtccaacatcaccctgccaatgcaggacaacaacaccgacgtctactgcatcagaagcaaccagttctccgtgtacgtccactccacctgcaagtcctccctctgggacaacatcttcaaccaggactgcacagacgtgctggaggccacagctgtgatcaagacaggaacctgccctttctcattcgacaagctcaacaactacctgaccttcaacaagttctgcctgagcctgtccccagtgggagccaactgcaagttcgacgtggccgccagaaccaggaccaacgagcaggtggtcagaagcctgtacgtcatctacgaggagggagacaacatcgtgggagtgcccagcgacaactcaggcctgcacgacctgagcgtgctgcacctggactcctgcacagactacaacatctacggcaggacaggagtgggcatcatcaggaggaccaacagcacactgctgtccggcctctactacacctccctgtccggagacttgctgggattcaagaacgtgtcagacggagtcatctacagcgtcaccccatgtgacgtgagcgcccaggcagcagtgatagacggagccatcgtgggagccatgacctcaatcaactcagaactgctgggcctcacccactggacaacaacacccaacttctactactactccatctacaactacacatcagaaagaacaagggacacagcaatcgactccaacgacgtggactgtgagccagtcatcacctactccaacatcggcgtgtgcaagaacggagccctggtgttcatcaacgtcacccactcagacggcgacgtccagccaatctccacaggaaacgtcaccatccccaccaacttcaccatcagcgtgcaggtggagtacatgcaggtctacaccaccccagtctccatcgactgtgccaggtacgtgtgcaacggcaacccaagatgcaacaaactgctgacccagtacgtgagcgcctgccagaccatcgagcaggccctggccatgggcgccaggctggagaacatggaggtggacagcatgctctttgtgagcgagaacgccctgaagcttgccagcgtggaggccttcaacagcaccgaaaacctggactccatctacaaagagtggccctccataggaggctcctggctgggaggcctgaaggacatcctcccatcccacaacagcaaaagaaagtacggcagcgccatcgaagacctgctgttcgacaaggtggtcacctcaggactgggcacagtggacgaggactacaagaggtgcaccggaggctacgacatcgcagacctggtctgtgcccagtactacaacggcatcatggtgctcccaggcgtggccaacgccgacaagatgaccatgtacacagcaagcctggctggaggaatcacactgggagccctgggaggaggggccgtggccattccattcgccgtggccgtgcaggccagactgaactacgtggccctgcagacagacgtgctaaacaagaaccagcagatcctggccaacgccttcaaccaggccatcggcaacatcacccaggccttcggcaaggtgaacgacgcaatccaccagacatcacagggcctggcaacagtggccaaggccctggccaaggtccaggacgtggtgaacacccagggccaggccctctcacacctgacagtccagctgcagaacaacttccaggcaatctcctcctccatctcagacatctacaacagactggaccccccctcagccgacgcccaggtggacagactcatcacaggcaggctgaccgccctcaacgccttcgtgtcccagaccctcaccaggcaggccgaggtgagggccagcaggcagctcgccaaggacaaggtgaacgagtgcgtcagaagccagagccagaggttcggcttctgtggcaacggcacccacctgttctccctggccaacgcagcccccaacggcatgatcttcttccacacagtcctcctcccaacagcatatgagacagtcaccgcctggtcaggaatctgtgcctcagacggggacagaaccttcggcctggtggtcaaggacgtgcagctgacactcttcagaaacctggacgacaaattctacctgacccccaggaccatgtaccagccaagggtggccacctcctcagacttcgtgcagatcgagggctgtgacgtgctcttcgtgaacgccaccgtcatcgacctcccatccatcatcccagactacatcgacatcaaccagacagtgcaggacatcctggagaactaccgccccaactggaccgtgccagagttcaccctagacatattcaacgccacctacctgaacctgacaggagaaattgacgacctggagttcagatcagaaaagctacacaacaccaccgtggagttagccatcctcatagacaacattaacaacaccctcgtcaacctggagtggctcaacaggattgaaacctacgtgaagtggccctggtacgtctggctcctcatcggcctggtggtggtcttctgcatcccactgctgctgttctgctgcttctccaccggctgctgtggatgcatcggctgcctgggctcatgctgccactcaatctgctcaaggaggcagtttgaaaactacgagccaatagaaaaagtccacgtccac

SEQ ID NO: 15 - DNA, 4299 bp, synthetic construct
  source 1..4299: mol_type = other DNA
accacaaataacgagtgcattcaggtcaacgtcacccagctggccggtaacgagaacctaattagagacttcctattctcgaactttaaagaggaaggctctgtggtggtcggaggttactaccccacagaagtgtggtacaattgctcacgtacagccaggaccactgccttccagtacttcaacaacattcatgccttctactttgtcatggaagccatggagaactccactgggaatgccagaggaaagcctctcctcttccatgtccatggagagcctgtctctgtgattatctcagcatatagggatgatgtgcagcagcggccgctgcttaagcatggcctagtgtgcattactaagaaccgacatatcaattatgagcagttcacctccaaccagtggaactccacatgcactggtgctgataggaagatcccgttcagcgttatccccaccgataatggcacaaagatttatggcctagaatggaacgatgattttgttactgcctacatatcaggaagaagttaccacttaaacattaacaccaattggttcaataatgttacacttctgtactctcgcagcagtacggccacttgggagtattcggctgcatatgcctaccaaggtgtaagcaacttcacctactacaagctgaacaatacgaacggtctgaagacttatgagctgtgcgaagactacgagcactgtacgggctatgcgacaaatgtcttcgccccgacgagcggcgggtacataccggatggcttctccttcaacaactggttcctccttaccaatagctccactttcgtatcaggaagatttgttacgaaccaaccccttctcattaactgtctgtggccagtgccctccttcggagtagctgctcaagagttctgtttcgagggtgcacagttcagccagtgtaatggagtgtcgctgaacaacactgtggacgtgatcaggtttaatttgaacttcacagctgatgttcagtccggcatgggcgcgactgtgttcagcctaaacaccacgggtggcgtcatcttggagattagttgttactctgacactgtgtcagagagcagcagttactcctacggagaaattcctttcggcatcacagacggtccccggtactgctatgtgctgtacaacggaactgctttgaagtacctggggacattgccaccttctgtgaaggaaatagccatctctaagtggggtcacttttacattaacggctataatttcttttccactttcccaattggatgcattagcttcaacctgacaacaggtgtgtctggagccttctggaccatcgcctatacctcttacacagaggctctagtacaggtggagaacacagctataaagaacgtgacgtactgtaacagtcacataaacaatatcaagtgttctcagttgactgcgaacttaaacaatgggttttatccagtggcgagctcggaggtggggtttgtaaacaaatctgtggtgctgttgccctccttcttcacgtacactgcagtgaacatcaccattgatttggggatgaaactgtccggctacgggcagcctatagcatctacactgagcaatatcacactgcccatgcaggataacaatacagatgtgtactgtatccgctcaaaccagttctctgtatacgtgcacagtacatgcaagagctcgctatgggacaacattttcaaccaggattgtactgatgtgcttgaagcaactgcagtgatcaaaacaggcacatgcccgttcagctttgataagctcaacaactacctaacgttcaacaagttctgcttgagcctgtctccagtaggcgccaattgcaagtttgacgttgcagcgcgaacacggacaaacgaacaggtagtgcggtcgctctatgttatctacgaggagggggacaacatagtcggggttccatccgacaactcaggtttgcacgacctgagtgtgctccatttggactcatgcacggattataacatctacgggcgcacaggtgtggggataatacgaagaacaaactctacgctattgagcgggctctactacacctcattgagtggggacctgctagggttcaagaacgtatctgacggtgtgatctatagcgtcacaccatgtgacgtatcagcccaagctgctgtgattgacggggcgattgtgggggctatgacttcaattaacagcgagctcctaggcctgacccactggactaccaccccaaacttctactactacagcatttataactataccagtgagcgcaccagggacactgccattgacagcaatgacgtcgactgcgagcctgttattacctacagcaacatcggtgtttgtaagaatggagctctagtcttcataaacgtaacgcactctgatggcgatgttcaaccaatttccactgggaacgtaaccatacccaccaactttactatttccgtccaggtggagtacatgcaagtatataccacgccagtgtccatcgactgcgctcggtatgtgtgcaacggtaacccacgctgcaataagctgctaacgcagtacgtcagcgcctgccagacaatagagcaggcattggcaatgggtgcaaggcttgaaaacatggaggtggactccatgttgttcgtgtctgaaaacgctcttaaactagcatccgtggaggcattcaacagtactgagaacttggactctatctataaggagtggccctccattgggggcagctggcttggaggtctaaaagacatcctgcccagccacaactccaagaggaagtacgggtccgctatagaggacctcctctttgacaaggttgttacttctggtcttggcacagtggacgaagactacaagaggtgcacaggaggctatgatatagctgacctggtgtgtgctcaatactacaacggtataatggttctcccaggtgtggccaacgctgacaagatgacaatgtacacagcctctttagctggaggcattaccctgggagcccttgggggtggcgcagtggcaattccatttgccgttgcggtgcaggcccgactaaactatgtcgcacttcaaacagatgtgctcaacaagaaccaacaaatactggccaacgctttcaaccaggccattggtaacattacgcaggcatttggcaaggtgaatgacgccatccaccagaccagccagggacttgccacagtggccaaggccttggcaaaggtgcaggatgtcgtgaacacacagggtcaggccctctctcatttgacagtgcagcttcagaataacttccaagcaatcagttcaagcatcagcgacatctacaaccggctggaccccccatctgcagatgcgcaggtggacaggctaatcactggacgcttgacggcactaaatgcctttgtcagccaaactctgacccggcaagcagaggtgcgggccagtagacaactggccaaagacaaggtcaacgagtgcgtcaggtcccagtcccagcgttttggattctgtgggaacgggacgcacctgttctcattagccaatgctgcacccaatggcatgatctttttccatactgttctacttcctactgcctatgaaaccgtgaccgcttggagcggcatctgcgcatctgatggcgataggaccttcgggctggtcgttaaggatgtccagctaacgctgttccggaacttggatgacaagttctacctgacccccaggaccatgtaccagccgagagtggcaacgagttctgacttcgtgcaaattgagggctgtgacgtcctgtttgttaatgcaacagtgatcgatctgcccagtatcataccagattacatagacataaaccagacagtccaggacatactggagaattacaggccaaactggaccgtaccagagttcacgctggacatattcaacgctacgtacctcaatttgactggggaaattgatgacttggagttcaggtcggagaagctccacaacaccactgtggagctggccatcctgattgacaacatcaacaacactctggtgaacctggagtggctaaatcgcattgaaacctatgtcaagtggccttggtacgtttggctactgatcggactcgtggtagtcttctgcataccactcctgctattttgctgcttcagcacagggtgctgtggctgcattggatgcctaggttcctgctgtcacagtatctgcagcagaagacaattcgagaactacgagcccatagaaaaggtccacgtacat

SEQ ID NO: 16 - protein, 26 aa, synthetic construct
MRFVMSPTVLLLLLGALAAPQTWAGS

SEQ ID NO: 17 - DNA, 78 bp, synthetic construct
  source 1..78: mol_type = other DNA
atgagatttgtgatgtcccccactgtcctgctgctgctcctgggagccctggcagccccccagacctgggcaggcagc

SEQ ID NO: 18 - DNA, 78 bp, synthetic construct
  source 1..78: mol_type = other DNA
atgagatttgtgatgagccccactgtgctgctgctgctgctgggagccctggcagccccccagacctgggctggctcc

SEQ ID NO: 19 - DNA, 78 bp, synthetic construct
  source 1..78: mol_type = other DNA
atgcgattcgtcatgtcaccaaccgttttactattattactaggagcattagcagcaccgcaaacatgggcaggaagt

SEQ ID NO: 20 - DNA, 78 bp, synthetic construct
  source 1..78: mol_type = other DNA
atgagattcgtgatgtcccctaccgtactactactcctacttggcgcactagcagctcctcaaacttgggccggatcc

SEQ ID NO: 21 - DNA, 78 bp, synthetic construct
  source 1..78: mol_type = other DNA
atgagatttgtgatgagccccactgtgctgctgctgctgctgggagccctggcagccccccagacctgggctggctca

SEQ ID NO: 22 - DNA, 78 bp, synthetic construct
  source 1..78: mol_type = other DNA
atgcgttttgtaatgtcacctactgtactactactactactcggagcactagcagcacctcagacttgggccggatca

SEQ ID NO: 23 - protein, 55 aa, synthetic construct
FLGIIAGVVVLVVTVVVGAVIWRKKCSGRKGPSYSHAARDDSTQGSDSSLMAPKV

SEQ ID NO: 24 - DNA, 165 bp, synthetic construct
  source 1..165: mol_type = other DNA
ttcctgggcatcatcgcaggagtggtggtgctggtggtgaccgtggtggtgggggctgtaatctggaggaagaagtgctcagggagaaagggcccaagctactctcacgccgccagggatgactccacacagggctcagactcctcactgatggctccaaaggtc

SEQ ID NO: 25 - DNA, 165 bp, synthetic construct
  source 1..165: mol_type = other DNA
ttcctgggcatcatcgcaggagtggtggtcctggtggtcacagtcgtggtgggagcagtgatctggaggaagaagtgctcaggaaggaagggcccatcctactcccacgccgccagggacgactcaacccagggctcagacagctccctgatggcccccaaggtg

SEQ ID NO: 26 - DNA, 165 bp, synthetic construct
  source 1..165: mol_type = other DNA
ttcctgggcatcatcgctggcgtggtggtcctggtggtgactgtggtggtcggagccgtcatctggaggaagaagtgcagcggcagaaagggcccaagctacagccacgccgccagagatgacagcacccagggcagcgacagcagcctcatggcccccaaggtc

SEQ ID NO: 27 - DNA, 165 bp, synthetic construct
  source 1..165: mol_type = other DNA
ttcctgggcatcatcgcaggagtggtggtgctggtggtgacagtggtggtgggagcagtgatctggagaaagaaatgcagcgggagaaagggccccagctacagccacgccgccagggacgacagcacccagggcagcgacagcagcctcatggcccccaaggtg

SEQ ID NO: 28 - DNA, 165 bp, synthetic construct
  source 1..165: mol_type = other DNA
ttcctgggcatcatcgccggcgtggtggtcctggtggtgaccgtggtggtcggagcagtgatctggaggaagaagtgctcaggcaggaagggcccatcctacagccacgccgccagagatgacagcacccaaggctcagacagctccctgatggcccccaaggtg

SEQ ID NO: 29 - DNA, 165 bp, synthetic construct
  source 1..165: mol_type = other DNA
ttccttggaatcatagctggggtcgttgtcctcgtagtgactgtagtggtaggcgcagttatctggaggaagaaatgctcggggaggaaagggccctcttacagccatgctgccagggatgactccacacaggggtcagatagcagcctcatggccccaaaggtc

SEQ ID NO: 30 - DNA, 165 bp, synthetic construct
  source 1..165: mol_type = other DNA
ttcctgggcatcatcgccggcgtggtggtcctggtggtcacagtggtggtgggagctgtgatctggagaaagaagtgcagcggcaggaagggcccaagctacagccacgctgccagagatgactccacccagggcagcgacagcagcctgatggcccccaaggtg

SEQ ID NO: 31 - DNA, 165 bp, synthetic construct
  source 1..165: mol_type = other DNA
ttcctgggcataatcgccggcgtggtggtgctggtggtcacagtggtggtcggagcagtgatctggaggaagaagtgctcagggaggaagggcccatcctactcccacgccgccagggacgacagcacccagggctcagactcatccctgatggcccccaaggtg

SEQ ID NO: 32 - DNA, 165 bp, synthetic construct
  source 1..165: mol_type = other DNA
ttcctggggataatcgcaggagtggttgttctagtggtgaccgtggtagttggggcagtgatctggagaaagaaatgctctggccgtaagggaccatcctactcccatgcagcacgtgatgattctacccagggcagcgacagttcattgatggcccctaaagtc

SEQ ID NO: 33 - protein, 27 aa, synthetic construct
YPYDVPDYAYPYDVPDYAYPYDVPDYA

SEQ ID NO: 34 - DNA, 81 bp, synthetic construct
  source 1..81: mol_type = other DNA
tacccctacgatgtgccagactacgcctacccctacgatgtgccagactacgcctacccctacgatgtgccagactacgcc

SEQ ID NO: 35 - DNA, 81 bp, synthetic construct
  source 1..81: mol_type = other DNA
tacccctacgacgtgcccgactacgcctacccctacgacgtgccagactacgcctacccctacgacgtgccagactacgcc

SEQ ID NO: 36 - DNA, 81 bp, synthetic construct
  source 1..81: mol_type = other DNA
tacccatacgatgttccagactacgcttacccatatgacgtgccagactatgcctacccctacgacgtgcccgactacgca

SEQ ID NO: 37 - protein, 6 aa, synthetic construct
HHHHHH

SEQ ID NO: 38 - DNA, 18 bp, synthetic construct
  source 1..18: mol_type = other DNA
caccaccaccaccaccac

SEQ ID NO: 39 - DNA, 18 bp, synthetic construct
  source 1..18: mol_type = other DNA
catcatcatcatcaccac

SEQ ID NO: 40 - protein, 24 aa, synthetic construct
DYKDDDDKDYKDDDDKDYKDDDDK

SEQ ID NO: 41 - DNA, 72 bp, synthetic construct
  source 1..72: mol_type = other DNA
gactacaaagatgatgatgacaaggactacaaagacgacgacgacaaagactacaaggacgatgacgacaag

SEQ ID NO: 42 - DNA, 72 bp, synthetic construct
  source 1..72: mol_type = other DNA
gactacaaggatgatgatgacaaggactacaaagacgacgacgacaaggactacaaggatgacgatgacaag

SEQ ID NO: 43 - DNA, 72 bp, synthetic construct
  source 1..72: mol_type = other DNA
gactataaagacgacgatgacaaagattataaagatgatgacgacaaggactacaaggatgatgatgacaag

SEQ ID NO: 44 - DNA, 741 bp, synthetic construct
  source 1..741: mol_type = other DNA
ttaaaacagcctgtgggttgatcccacccacaggcccattgggcgctagcactctggtatcacggtacctttgtgcgcctgttttataccccctcccccaactgtaacttagaagtaacacacaccgatcaacagtcagcgtggcacaccagccacgttttgatcaagcacttctgttaccccggactgagtatcaatagactgctcacgcggttgaaggagaaagcgttcgttatccggccaactacttcgaaaaacctagtaacaccgtggaagttgcagagtgtttcgctcagcactaccccagtgtagatcaggtcgatgagtcaccgcattccccacgggcgaccgtggcggtggctgcgttggcggcctgcccatggggaaacccatgggacgctctaatacagacatggtgcgaagagtctattgagctagttggtagtcctccggcccctgaatgcggctaatcctaactgcggagcacacaccctcaagccagagggcagtgtgtcgtaacgggcaactctgcagcggaaccgactactttgggtgtccgtgtttcattttattcctatactggctgcttatggtgacaattgagagatcgttaccatatagctattggattggccatccggtgactaatagagctattatatatccctttgttgggtttataccacttagcttgaaagaggttaaaacattacaattcattgttaagttgaatacagcaaa

SEQ ID NO: 45 - protein, 26 aa, synthetic construct
RAKRGSGATNFSLLKQAGDVEENPGP

SEQ ID NO: 46 - DNA, 78 bp, synthetic construct
  source 1..78: mol_type = other DNA
agagccaagagaggcagcggagccaccaacttcagcctgctgaagcaggccggcgacgtggaggagaacccaggacct

SEQ ID NO: 47 - protein, 15 aa, synthetic construct
GGGGSGGGGSGGGGS

SEQ ID NO: 48 - DNA, 45 bp, synthetic construct
  source 1..45: mol_type = other DNA
ggaggaggaggaagcggaggaggaggaagcggaggaggaggaagc